European Patent Specification EP 3 904 388 B1, published May 6, 2026. Title: FUCOSIDASE FROM BACTEROIDES AND METHODS USING THE SAME. Applicant: ACADEMIA SINICA. The sequence listing filed with the application follows.

SEQUENCE LISTING (19 sequences)

SEQ ID NO: 1 - protein, 414 aa, Bacteroides sp.
QQKYQPTEANLKARSEFQDNKFGIFLHWGLYAMLATGEWTMTNNNLNYKEYAKLAGGFYPSKFDADKWVAAIKASGAKYICFTTRHHEGFSMFDTKYSDYNIVKATPFKRDVVKELADACAKHGIKLHFYYSHIDWYREDAPQGRTGRRTGRPNPKGDWKSYYQFMNNQLTELLTNYGPIGAIWFDGWWDQDINPDFDWELPEQYALIHRLQPACLVGNNHHQTPFAGEDIQIFERDLPGENTAGLSGQSVSHLPLETCETMNGMWGYKITDQNYKSTKTLIHYLVKAAGKDANLLMNIGPQPDGELPEVAVQRLKEVGEWMSKYGETIYGTRGGLVAPHDWGVTTQKGNKLYVHILNLQDKALFLPIVDKKVKKAVVFADKTPVRFTKNKEGIVLELAKVPTDVDYVVELTID

SEQ ID NO: 2 - protein, 414 aa, Bacteroides sp.
QSSYQPGEENLKAREEFQDNKFGIFLHWGLYAMLATGEWTMTNNNLNYKEYAKLAGGFYPSKFDADKWVAAIKASGAKYICLTSRHHDGFSMFDTQYSDFNIVKATPFKRDIIKELAAACSKQGIKLHFYYSHLDWTREDYPWGRTGRGTGRSNPQGDWKSYYQFMNNQLTELLTNYGPVGAIWFDGWWDQDGNPGFNWELPEQYAMIHKLQPGCLIGNNHHQTPFAGEDIQIFERDLPGENTAGLSGQSVSHLPLETCETMNGMWGYKITDQNYKSTKTLIHYLVKAAGKNANLLMNIGPQPDGELPEVAVQRLKEMGEWMNQYGETIYGTRGGAVAPHDWGVTTQKGNKLYVHILNLQDKALFLPLADKKVKKAVLFKNGTPVRFTKNKEGVLLEFTEIPKDIDYVVELTID

SEQ ID NO: 3 - DNA, 38 bp, Artificial Sequence
  Description of Artificial Sequence: Synthetic primer
ttcagggagcgatcgctcagcaaaagtatcaaccgaca

SEQ ID NO: 4 - DNA, 39 bp, Artificial Sequence
  Description of Artificial Sequence: Synthetic primer
gtcattacgtttaaacttagtcaattgtaagttctacca

SEQ ID NO: 5 - DNA, 38 bp, Artificial Sequence
  Description of Artificial Sequence: Synthetic primer
ttcagggagcgatcgctcagtcttcttaccagcctggt

SEQ ID NO: 6 - DNA, 40 bp, Artificial Sequence
  Description of Artificial Sequence: Synthetic primer
gtcattacgtttaaacttagtcaattgtaagttctacaac

SEQ ID NO: 7 - DNA, 36 bp, Artificial Sequence
  Description of Artificial Sequence: Synthetic primer
ttcagggagcgatcgctgcggttaccggtaccacca

SEQ ID NO: 8 - DNA, 39 bp, Artificial Sequence
  Description of Artificial Sequence: Synthetic primer
gtcattacgtttaaacttaccagtctttagagtacgggg

SEQ ID NO: 9 - DNA, 38 bp, Artificial Sequence
  Description of Artificial Sequence: Synthetic primer
tttcagggagcgatcgctgcggttaacctgtctaacct

SEQ ID NO: 10 - DNA, 40 bp, Artificial Sequence
  Description of Artificial Sequence: Synthetic primer
gtcattacgtttaaacttacgggttcatgattttgatcag

SEQ ID NO: 11 - DNA, 36 bp, Artificial Sequence
  Description of Artificial Sequence: Synthetic primer
ttcagggagcgatcgctgcgaccgcgctggcgggtt

SEQ ID NO: 12 - DNA, 40 bp, Artificial Sequence
  Description of Artificial Sequence: Synthetic primer
gtcattacgtttaaacttagtttttaaccgcgtcacgaac

SEQ ID NO: 13 - DNA, 37 bp, Artificial Sequence
  Description of Artificial Sequence: Synthetic primer
ttcagggagcgatcgctgcgccggcgccggttaaaca

SEQ ID NO: 14 - DNA, 39 bp, Artificial Sequence
  Description of Artificial Sequence: Synthetic primer
gtcattacgtttaaacttacggggtacgaaccgcttcag

SEQ ID NO: 15 - DNA, 38 bp, Artificial Sequence
  Description of Artificial Sequence: Synthetic primer
ttcagggagcgatcgctacccaccatgattcactcaat

SEQ ID NO: 16 - DNA, 41 bp, Artificial Sequence
  Description of Artificial Sequence: Synthetic primer
gtcattacgtttaaacttatttttttagcagctgccttttc

SEQ ID NO: 17 - DNA, 37 bp, Artificial Sequence
  Description of Artificial Sequence: Synthetic primer
ttcagggagcgatcgctgcgccggcggacaacaccgt

SEQ ID NO: 18 - DNA, 40 bp, Artificial Sequence
  Description of Artificial Sequence: Synthetic primer
gtcattacgtttaaacttagttggtaacaaccggcgcaga

SEQ ID NO: 19 - protein, 6 aa, Artificial Sequence
  Description of Artificial Sequence: Synthetic 6xHis Tag
HHHHHH